European Patent Specification EP 3 234 150 B1, published August 13, 2025. Title: FUNGAL GENOME MODIFICATION SYSTEMS AND METHODS OF USE. Applicant: DANISCO US INC. Ward, Michael Chan, Jimmy Bower, Benjamin S. Madrid, Susan Mampusti Ge, Jing Gu, Xiaogang Song, Danfeng Song, Mingmin. The sequence listing filed with the application follows.

SEQUENCE LISTING (81 sequences)

SEQ ID NO: 1 - DNA, 842 bp, T. reesei
aaaaaacactagtaagtacttacttatgtattattaactactttagctaacttctgcagtactacctaagaggctaggggtagttttatagcagacttatagctattatttttatttagtaaagtgcttttaaagtaaggtcttttttatagcactttttatttattataatatatattatataataattttaagcctggaatagtaaagaggcttatataataatttatagtaataaaagcttagcagctgtaatataattcctaaagaaacagcatgaaatggtattatgtaagagctatagtctaaaggcactctgctggataaaaatagtggctataagtctgctgcaaaactacccccaacctcgtaggtatataagtactgtttgatggtagtctatcgccttcgggcatttggtcaatttataacgatacaggttcgtttcggcttttcctcggaacccccagaggtcatcagttcgaatcgctaacaggtcaacagagaagattagcatggcccctgcactaaggatgacacgctcactcaaagagaagctaaacattttttttctcttccaagtcgtgatggttatctttttgcttagagaatctattcttgtggacgattagtattggtaaatccctgctgcacattgcggcggatggtctcaacggcataataccccattcgtgatgcagcggtgatcttcaatatgtagtgtaatacgttgcatacaccaccaggttcggtgcctcctgtatgtacagtactgtagttcgactcctccgcgcaggtggaaacgattccctagtgggcaggtattttggcggggtcaagaa

SEQ ID NO: 2 - RNA, 99 nt, Artificial Sequence
  Synthetic sequence
  misc_feature (1)..(20): n is a, c, g, or u
nnnnnnnnnnnnnnnnnnnnguuuuagagcuagaaauagcaaguuaaaauaaggcuaguccguuaucaacuugaaaaaguggcaccgagucgguggugc

SEQ ID NO: 3 - RNA, 99 nt, Artificial Sequence
  Synthetic sequence
guccucgagcaaaaggugccguuuuagagcuagaaauagcaaguuaaaauaaggcuaguccguuaucaacuugaaaaaguggcaccgagucgguggugc

SEQ ID NO: 4 - RNA, 99 nt, Artificial Sequence
  Synthetic sequence
guucagugcaauaggcgucuguuuuagagcuagaaauagcaaguuaaaauaaggcuaguccguuaucaacuugaaaaaguggcaccgagucgguggugc

SEQ ID NO: 5 - RNA, 99 nt, Artificial Sequence
  Synthetic sequence
gccaauggcgacggcagcacguuuuagagcuagaaauagcaaguuaaaauaaggcuaguccguuaucaacuugaaaaaguggcaccgagucgguggugc

SEQ ID NO: 6 - RNA, 99 nt, Artificial Sequence
  Synthetic sequence
gcacagcgggaugcccuuguguuuuagagcuagaaauagcaaguuaaaauaaggcuaguccguuaucaacuugaaaaaguggcaccgagucgguggugc

SEQ ID NO: 7 - DNA, 4155 bp, Artificial Sequence
  codon optimized seqs
atggcaccgaagaagaagcgcaaggtgatggacaagaagtacagcatcggcctcgacatcggcaccaactcggtgggctgggccgtcatcacggacgaatataaggtcccgtcgaagaagttcaaggtcctcggcaatacagaccgccacagcatcaagaaaaacttgatcggcgccctcctgttcgatagcggcgagaccgcggaggcgaccaggctcaagaggaccgccaggagacggtacactaggcgcaagaacaggatctgctacctgcaggagatcttcagcaacgagatggcgaaggtggacgactccttcttccaccgcctggaggaatcattcctggtggaggaggacaagaagcatgagcggcacccaatcttcggcaacatcgtcgacgaggtggcctaccacgagaagtacccgacaatctaccacctccggaagaaactggtggacagcacagacaaggcggacctccggctcatctaccttgccctcgcgcatatgatcaagttccgcggccacttcctcatcgagggcgacctgaacccggacaactccgacgtggacaagctgttcatccagctcgtgcagacgtacaatcaactgttcgaggagaaccccataaacgctagcggcgtggacgccaaggccatcctctcggccaggctctcgaaatcaagaaggctggagaaccttatcgcgcagttgccaggcgaaaagaagaacggcctcttcggcaaccttattgcgctcagcctcggcctgacgccgaacttcaaatcaaacttcgacctcgcggaggacgccaagctccagctctcaaaggacacctacgacgacgacctcgacaacctcctggcccagataggagaccagtacgcggacctcttcctcgccgccaagaacctctccgacgctatcctgctcagcgacatccttcgggtcaacaccgaaattaccaaggcaccgctgtccgccagcatgattaaacgctacgacgagcaccatcaggacctcacgctgctcaaggcactcgtccgccagcagctccccgagaagtacaaggagatcttcttcgaccaatcaaaaaacggctacgcgggatatatcgacggcggtgccagccaggaagagttctacaagttcatcaaaccaatcctggagaagatggacggcaccgaggagttgctggtcaagctcaacagggaggacctcctcaggaagcagaggaccttcgacaacggctccatcccgcatcagatccacctgggcgaactgcatgccatcctgcggcgccaggaggacttctacccgttcctgaaggataaccgggagaagatcgagaagatcttgacgttccgcatcccatactacgtgggcccgctggctcgcggcaactcccggttcgcctggatgacccggaagtcggaggagaccatcacaccctggaactttgaggaggtggtcgataagggcgctagcgctcagagcttcatcgagcgcatgaccaacttcgataaaaacctgcccaatgaaaaagtcctccccaagcactcgctgctctacgagtacttcaccgtgtacaacgagctcaccaaggtcaaatacgtcaccgagggcatgcggaagccggcgttcctgagcggcgagcagaagaaggcgatagtggacctcctcttcaagaccaacaggaaggtgaccgtgaagcaattaaaagaggactacttcaagaaaatagagtgcttcgactccgtggagatctcgggcgtggaggatcggttcaacgcctcactcggcacgtatcacgacctcctcaagatcattaaagacaaggacttcctcgacaacgaggagaacgaggacatcctcgaggacatcgtcctcaccctgaccctgttcgaggaccgcgaaatgatcgaggagaggctgaagacctacgcgcacctgttcgacgacaaggtcatgaaacagctcaagaggcgccgctacactggttggggaaggctgtcccgcaagctcattaatggcatcagggacaagcagagcggcaagaccatcctggacttcctcaagtccgacgggttcgccaaccgcaacttcatgcagctcattcacgacgactcgctcacgttcaaggaagacatccagaaggcacaggtgagcgggcagggtgactccctccacgaacacatcgccaacctggccggctcgccggccattaaaaagggcatcctgcagacggtcaaggtcgtcgacgagctcgtgaaggtgatgggccggcacaagcccgaaaatatcgtcatagagatggccagggagaaccagaccacccaaaaagggcagaagaactcgcgcgagcggatgaaacggatcgaggagggcattaaagagctcgggtcccagatcctgaaggagcaccccgtggaaaatacccagctccagaatgaaaagctctacctctactacctgcagaacggccgcgacatgtacgtggaccaggagctggacattaatcggctatcggactacgacgtcgaccacatcgtgccgcagtcgttcctcaaggacgatagcatcgacaacaaggtgctcacccggtcggataaaaatcggggcaagagcgacaacgtgcccagcgaggaggtcgtgaagaagatgaaaaactactggcgccagctcctcaacgcgaaactgatcacccagcgcaagttcgacaacctgacgaaggcggaacgcggtggcttgagcgaactcgataaggcgggcttcataaaaaggcagctggtcgagacgcgccagatcacgaagcatgtcgcccagatcctggacagccgcatgaatactaagtacgatgaaaacgacaagctgatccgggaggtgaaggtgatcacgctgaagtccaagctcgtgtcggacttccgcaaggacttccagttctacaaggtccgcgagatcaacaactaccaccacgcccacgacgcctacctgaatgcggtggtcgggaccgccctgatcaagaagtacccgaagctggagtcggagttcgtgtacggcgactacaaggtctacgacgtgcgcaaaatgatcgccaagtccgagcaggagatcggcaaggccacggcaaaatacttcttctactcgaacatcatgaacttcttcaagaccgagatcaccctcgcgaacggcgagatccgcaagcgcccgctcatcgaaaccaacggcgagacgggcgagatcgtctgggataagggccgggatttcgcgacggtccgcaaggtgctctccatgccgcaagtcaatatcgtgaaaaagacggaggtccagacgggcgggttcagcaaggagtccatcctcccgaagcgcaactccgacaagctcatcgcgaggaagaaggattgggacccgaaaaaatatggcggcttcgacagcccgaccgtcgcatacagcgtcctcgtcgtggcgaaggtggagaagggcaagtcaaagaagctcaagtccgtgaaggagctgctcgggatcacgattatggagcggtcctccttcgagaagaacccgatcgacttcctagaggccaagggatataaggaggtcaagaaggacctgattattaaactgccgaagtactcgctcttcgagctggaaaacggccgcaagaggatgctcgcctccgcaggcgagttgcagaagggcaacgagctcgccctcccgagcaaatacgtcaatttcctgtacctcgctagccactatgaaaagctcaagggcagcccggaggacaacgagcagaagcagctcttcgtggagcagcacaagcattacctggacgagatcatcgagcagatcagcgagttctcgaagcgggtgatcctcgccgacgcgaacctggacaaggtgctgtcggcatataacaagcaccgcgacaaaccaatacgcgagcaggccgaaaatatcatccacctcttcaccctcaccaacctcggcgctccggcagccttcaagtacttcgacaccacgattgaccggaagcggtacacgagcacgaaggaggtgctcgatgcgacgctgatccaccagagcatcacagggctctatgaaacacgcatcgacctgagccagctgggcggagacaagaagaagaagctcaagctctag

SEQ ID NO: 8 - protein, 1384 aa, Artificial Sequence
  protein expressed from synthetic construct
MAPKKKRKVMDKKYSIGLDIGTNSVGWAVITDEYKVPSKKFKVLGNTDRHSIKKNLIGALLFDSGETAEATRLKRTARRRYTRRKNRICYLQEIFSNEMAKVDDSFFHRLEESFLVEEDKKHERHPIFGNIVDEVAYHEKYPTIYHLRKKLVDSTDKADLRLIYLALAHMIKFRGHFLIEGDLNPDNSDVDKLFIQLVQTYNQLFEENPINASGVDAKAILSARLSKSRRLENLIAQLPGEKKNGLFGNLIALSLGLTPNFKSNFDLAEDAKLQLSKDTYDDDLDNLLAQIGDQYADLFLAAKNLSDAILLSDILRVNTEITKAPLSASMIKRYDEHHQDLTLLKALVRQQLPEKYKEIFFDQSKNGYAGYIDGGASQEEFYKFIKPILEKMDGTEELLVKLNREDLLRKQRTFDNGSIPHQIHLGELHAILRRQEDFYPFLKDNREKIEKILTFRIPYYVGPLARGNSRFAWMTRKSEETITPWNFEEVVDKGASAQSFIERMTNFDKNLPNEKVLPKHSLLYEYFTVYNELTKVKYVTEGMRKPAFLSGEQKKAIVDLLFKTNRKVTVKQLKEDYFKKIECFDSVEISGVEDRFNASLGTYHDLLKIIKDKDFLDNEENEDILEDIVLTLTLFEDREMIEERLKTYAHLFDDKVMKQLKRRRYTGWGRLSRKLINGIRDKQSGKTILDFLKSDGFANRNFMQLIHDDSLTFKEDIQKAQVSGQGDSLHEHIANLAGSPAIKKGILQTVKVVDELVKVMGRHKPENIVIEMARENQTTQKGQKNSRERMKRIEEGIKELGSQILKEHPVENTQLQNEKLYLYYLQNGRDMYVDQELDINRLSDYDVDHIVPQSFLKDDSIDNKVLTRSDKNRGKSDNVPSEEVVKKMKNYWRQLLNAKLITQRKFDNLTKAERGGLSELDKAGFIKRQLVETRQITKHVAQILDSRMNTKYDENDKLIREVKVITLKSKLVSDFRKDFQFYKVREINNYHHAHDAYLNAVVGTALIKKYPKLESEFVYGDYKVYDVRKMIAKSEQEIGKATAKYFFYSNIMNFFKTEITLANGEIRKRPLIETNGETGEIVWDKGRDFATVRKVLSMPQVNIVKKTEVQTGGFSKESILPKRNSDKLIARKKDWDPKKYGGFDSPTVAYSVLVVAKVEKGKSKKLKSVKELLGITIMERSSFEKNPIDFLEAKGYKEVKKDLIIKLPKYSLFELENGRKRMLASAGELQKGNELALPSKYVNFLYLASHYEKLKGSPEDNEQKQLFVEQHKHYLDEIIEQISEFSKRVILADANLDKVLSAYNKHRDKPIREQAENIIHLFTLTNLGAPAAFKYFDTTIDRKRYTSTKEVLDATLIHQSITGLYETRIDLSQLGGDKKKKLKL

SEQ ID NO: 9 - DNA, 412 bp, Artificial Sequence
  Synthetic sequence
gaattcggatcctctttgaaaagataatgtatgattatgctttcactcatatttatacagaaacttgatgttttctttcgagtatatacaaggtgattacatgtacgtttgaagtacaactctagattttgtagtgccctcttgggctagcggtaaaggtgcgcattttttcacaccctacaatgttctgttcaaaagattttggtcaaacgctgtagaagtgaaagttggtgcgcatgtttcggcgttcgaaacttctccgcagtgaaagataaatgatcgtcctcgagcaaaaggtgccgttttagagctagaaatagcaagttaaaataaggctagtccgttatcaacttgaaaaagtggcaccgagtcggtggtgctttttttgttttttatgtctgaattcggatcc

SEQ ID NO: 10 - DNA, 540 bp, Artificial Sequence
  Synthetic sequence
gaattcggatccaaaaaacactagtaagtacttacttatgtattattaactactttagctaacttctgcagtactacctaagaggctaggggtagttttatagcagacttatagctattatttttatttagtaaagtgcttttaaagtaaggtcttttttatagcactttttatttattataatatatattatataataattttaagcctggaatagtaaagaggcttatataataatttatagtaataaaagcttagcagctgtaatataattcctaaagaaacagcatgaaatggtattatgtaagagctatagtctaaaggcactctgctggataaaaatagtggctataagtctgctgcaaaactacccccaacctcgtaggtatataagtactgtttgatggtagtctatcgtcctcgagcaaaaggtgccgttttagagctagaaatagcaagttaaaataaggctagtccgttatcaacttgaaaaagtggcaccgagtcggtggtgcttttttttctcttgaattcggatcc

SEQ ID NO: 11 - DNA, 597 bp, Artificial Sequence
  Synthetic sequence
gaattcggatccaaaaaacactagtaagtacttacttatgtattattaactactttagctaacttctgcagtactacctaagaggctaggggtagttttatagcagacttatagctattatttttatttagtaaagtgcttttaaagtaaggtcttttttatagcactttttatttattataatatatattatataataattttaagcctggaatagtaaagaggcttatataataatttatagtaataaaagcttagcagctgtaatataattcctaaagaaacagcatgaaatggtattatgtaagagctatagtctaaaggcactctgctggataaaaatagtggctataagtctgctgcaaaactacccccaacctcgtaggtatataagtactgtttgatggtagtctatcgtcctcgagcaaaaggtgccgttttagagctagagttcgtttcggcttttcctcggaacccccagaggtcatcagttcgaatcgctaacagaatagcaagttaaaataaggctagtccgttatcaacttgaaaaagtggcaccgagtcggtggtgcttttttttctcttgaattcggatcc

SEQ ID NO: 12 - DNA, 315 bp, Artificial Sequence
  Synthetic sequence
aattcctaaagaaacagcatgaaatggtattatgtaagagctatagtctaaaggcactctgctggataaaaatagtggctataagtctgctgcaaaactacccccaacctcgtaggtatataagtactgtttgatggtagtctatcgccaatggcgacggcagcacgttttagagctagagttcgtttcggcttttcctcggaacccccagaggtcatcagttcgaatcgctaacagaatagcaagttaaaataaggctagtccgttatcaacttgaaaaagtggcaccgagtcggtggtgcttttttttctctt

SEQ ID NO: 13 - DNA, 39 bp, Artificial Sequence
  Primer
cgtcagcttaagaattcctaaagaaacagcatgaaatgg

SEQ ID NO: 14 - DNA, 47 bp, Artificial Sequence
  Primer
cgtcagggccacgtgggccaagagaaaaaaaagcaccaccgactcgg

SEQ ID NO: 15 - DNA, 23 bp, Artificial Sequence
  Primer
tgaacacagccaccgacatcagc

SEQ ID NO: 16 - DNA, 23 bp, Artificial Sequence
  Primer
gctggtgagggtttgtgctattg

SEQ ID NO: 17 - DNA, 21 bp, Artificial Sequence
  Primer
gattgcttgggaggaggacat

SEQ ID NO: 18 - DNA, 23 bp, Artificial Sequence
  Primer
cgaggccactgatgaagttgttc

SEQ ID NO: 19 - DNA, 23 bp, Artificial Sequence
  Primer
cagttttccaaggctgccaacgc

SEQ ID NO: 20 - DNA, 22 bp, Artificial Sequence
  Primer
ctgatcttgcaccctggaaatc

SEQ ID NO: 21 - DNA, 23 bp, Artificial Sequence
  Primer
ctctctatcatttgccaccctcc

SEQ ID NO: 22 - DNA, 22 bp, Artificial Sequence
  Primer
ctccattcaccctcaattctcc

SEQ ID NO: 23 - DNA, 23 bp, Artificial Sequence
  Primer
gttcccttggcggtgcttggatc

SEQ ID NO: 24 - DNA, 23 bp, Artificial Sequence
  Primer
caatagcacaaaccctcaccagc

SEQ ID NO: 25 - DNA, 23 bp, Artificial Sequence
  Primer
gaacaacttcatcagtggcctcg

SEQ ID NO: 26 - DNA, 23 bp, Artificial Sequence
  Primer
ccgttagttgaagatccttgccg

SEQ ID NO: 27 - DNA, 23 bp, Artificial Sequence
  Primer
gtcgaggatttgcttcatacctc

SEQ ID NO: 28 - DNA, 23 bp, Artificial Sequence
  Primer
gagagacgcaggatgactcaaag

SEQ ID NO: 29 - DNA, 23 bp, Artificial Sequence
  Primer
tgccgtgggtcattggcatattc

SEQ ID NO: 30 - DNA, 23 bp, Artificial Sequence
  Primer
tgccgactttgtccagtgattcg

SEQ ID NO: 31 - DNA, 23 bp, Artificial Sequence
  Primer
ttacatgtggacgcgagatagcg

SEQ ID NO: 32 - DNA, 22 bp, Artificial Sequence
  Primer
gtgtgtctaatgcctccaccac

SEQ ID NO: 33 - DNA, 22 bp, Artificial Sequence
  Primer
gatcgtgctagcgctgctgttg

SEQ ID NO: 34 - DNA, 21 bp, Artificial Sequence
  Primer
ccgtgatggagcccgtcttct

SEQ ID NO: 35 - DNA, 22 bp, Artificial Sequence
  Primer
cgcggtgagttcaggctttttc

SEQ ID NO: 36 - DNA, 22 bp, Artificial Sequence
  Primer
gtataagagcaggaggagggag

SEQ ID NO: 37 - DNA, 22 bp, Artificial Sequence
  Primer
gaacgcctcaatcagtcagtcg

SEQ ID NO: 38 - DNA, 2431 bp, Artificial Sequence
  Synthetic sequence
tcaggaaatagctttaagtagcttattaagtattaaaattatatatatttttaatataactatatttctttaataaataggtattttaagctttatatataaatataataataaaataatatattatatagctttttattaataaataaaatagctaaaaatataaaaaaaatagctttaaaatacttatttttaattagaattttatatatttttaatatataagatcttttacttttttataagcttcctaccttaaattaaatttttacttttttttactattttactatatcttaaataaaggctttaaaaatataaaaaaaatcttcttatatattataagctataaggattatatatatatttttttttaatttttaaagtaagtattaaagctagaattaaagttttaattttttaaggctttatttaaaaaaaggcagtaatagcttataaaagaaatttctttttcttttatactaaaagtactttttttttaataaggttagggttagggtttactcacaccgaccatcccaaccacatcttagggttagggttagggttagggttagggttagggttagggttagggtaagggtttaaacaaagccacgttgtgtctcaaaatctctgatgttacattgcacaagataaaaatatatcatcatgaacaataaaactgtctgcttacataaacagtaatacaaggggtgttatgagccatattcaacgggaaacgtcttgctcgaggccgcgattaaattccaacatggatgctgatttatatgggtataaatgggctcgcgataatgtcgggcaatcaggtgcgacaatctatcgattgtatgggaagcccgatgcgccagagttgtttctgaaacatggcaaaggtagcgttgccaatgatgttacagatgagatggtcagactaaactggctgacggaatttatgcctcttccgaccatcaagcattttatccgtactcctgatgatgcatggttactcaccactgcgatccccgggaaaacagcattccaggtattagaagaatatcctgattcaggtgaaaatattgttgatgcgctggcagtgttcctgcgccggttgcattcgattcctgtttgtaattgtccttttaacagcgatcgcgtatttcgtctcgctcaggcgcaatcacgaatgaataacggtttggttgatgcgagtgattttgatgacgagcgtaatggctggcctgttgaacaagtctggaaagaaatgcataagcttttgccattctcaccggattcagtcgtcactcatggtgatttctcacttgataaccttatttttgacgaggggaaattaataggttgtattgatgttggacgagtcggaatcgcagaccgataccaggatcttgccatcctatggaactgcctcggtgagttttctccttcattacagaaacggctttttcaaaaatatggtattgataatcctgatatgaataaattgcagtttcatttgatgctcgatgagtttttctaatcagaattggttaattggttgtaacactggcagagcattacgctgacttgacgggacggcggctttgttgaataaatcgaacttttgctgagttgaaggatcagatcacgcatcttcccgacaacgcagaccgttccgtggcaaagcaaaagttcaaaatcaccaactggtccacctacaacaaagctctcatcaaccgtggctccctcactttctggctggatgatggggcgattcaggcctggtatgagtcagcaacaccttcttcacgaggcagacctcagcggtttaaacctaaccctaaccctaaccctaaccctaaccctaaccctaaccctaaccctaaccctaaccctaaccctaaccctaaccctaacctaaccctaatggggtcgatctgaaccgaggatgagggttctatagactaatctacaggccgtacatggtgtgattgcagatgcgacgggcaaggtgtacagtgtccagaaggaggagagcggcataggtattgtaatagaccagctttacataataatcgcctgttgctactgactgatgaccttcttccctaaccagtttcctaattaccactgcagtgaggataaccctaactcgctctggggttattattatactgattagcaggtggcttatatagtgctgaagtactataagagtttctgcgggaggaggtggaaggactataaactggacacagttagggatagagtgatgacaagacctgaatgttatcctccggtgtggtatagcgaattggctgaccttgcagatggtaatggtttaggcagggtttttgcagagggggacgagaacgcgttctgcgatttaacggctgctgccgccaagctttacggttctctaatgggcggccgc

SEQ ID NO: 39 - DNA, 982 bp, Artificial Sequence
  Synthetic sequence
gtgtgtctaatgcctccaccacaggaaccaaaccggctttgacctctgggaagaagtcaatgggagctcattctttactgttgccaaccagcaccgaggtatgaagcaaatcctcgacattcgctgctactgcacatgagcattgttactgaccagctctacagcacttgtcgagggcgccactcttgctgccactcttggccagtcgggaagcgcttattcatctgttgctccccaggttttgtgctttctccaacgattctgggtgtcgtctggtggatacgtcgactccaacagtatgtcttttcactgtttatatgagattggccaatactgatagctcgcctctagtcaacaccaacgagggcaggactggcaaggatgtcaactccgtcctgacttccatccacaccttcgatcccaaccttggctgtgacgcaggcaccttccagccatgcagtgacaaagcgctctccaacctcaaggttgttgtcgactccttccgctccatctacggcgtgaacaagggcattcctgcggtgctgccgtcgccattggccggtatgcagaggatgtgtactacaacggcaacccttggtatcttgctacatttgctgctgccgagcagctgtacgatgccatctacgtctggaagaagacgggctccatcacggtgaccgccacctccctggccttcttccaggagcttgttcctggcgtgacggccgggacctactccagcagctcttcgacctttaccaacatcatcaacgccgtctcgacatacgccgatggcttcctcagcgaggctgccaagtacgtccccgccgacggttcgctggccgagcagtttgaccgcaacagcggcactccgctgtctgcgcttcacctgacgtggtcgtacgcctcgttcttgacagccacggcccgtcgggctggcatcgtgcccccctcgtgggccaacagcagcgctagcacgatc

SEQ ID NO: 40 - DNA, 404 bp, T. reesei
aaaaaacactagtaagtacttacttatgtattattaactactttagctaacttctgcagtactacctaagaggctaggggtagttttatagcagacttatagctattatttttatttagtaaagtgcttttaaagtaaggtcttttttatagcactttttatttattataatatatattatataataattttaagcctggaatagtaaagaggcttatataataatttatagtaataaaagcttagcagctgtaatataattcctaaagaaacagcatgaaatggtattatgtaagagctatagtctaaaggcactctgctggataaaaatagtggctataagtctgctgcaaaactacccccaacctcgtaggtatataagtactgtttgatggtagtctatc

SEQ ID NO: 41 - DNA, 146 bp, T. reesei
aattcctaaagaaacagcatgaaatggtattatgtaagagctatagtctaaaggcactctgctggataaaaatagtggctataagtctgctgcaaaactacccccaacctcgtaggtatataagtactgtttgatggtagtctatc

SEQ ID NO: 42 - DNA, 57 bp, T. reesei
gttcgtttcggcttttcctcggaacccccagaggtcatcagttcgaatcgctaacag

SEQ ID NO: 43 - DNA, 13 bp, T. reesei
ttttttttctctt

SEQ ID NO: 44 - DNA, 4104 bp, Artificial Sequence
  codon optimized seqs
atggacaagaagtacagcatcggcctcgacatcggcaccaactcggtgggctgggccgtcatcacggacgaatataaggtcccgtcgaagaagttcaaggtcctcggcaatacagaccgccacagcatcaagaaaaacttgatcggcgccctcctgttcgatagcggcgagaccgcggaggcgaccaggctcaagaggaccgccaggagacggtacactaggcgcaagaacaggatctgctacctgcaggagatcttcagcaacgagatggcgaaggtggacgactccttcttccaccgcctggaggaatcattcctggtggaggaggacaagaagcatgagcggcacccaatcttcggcaacatcgtcgacgaggtggcctaccacgagaagtacccgacaatctaccacctccggaagaaactggtggacagcacagacaaggcggacctccggctcatctaccttgccctcgcgcatatgatcaagttccgcggccacttcctcatcgagggcgacctgaacccggacaactccgacgtggacaagctgttcatccagctcgtgcagacgtacaatcaactgttcgaggagaaccccataaacgctagcggcgtggacgccaaggccatcctctcggccaggctctcgaaatcaagaaggctggagaaccttatcgcgcagttgccaggcgaaaagaagaacggcctcttcggcaaccttattgcgctcagcctcggcctgacgccgaacttcaaatcaaacttcgacctcgcggaggacgccaagctccagctctcaaaggacacctacgacgacgacctcgacaacctcctggcccagataggagaccagtacgcggacctcttcctcgccgccaagaacctctccgacgctatcctgctcagcgacatccttcgggtcaacaccgaaattaccaaggcaccgctgtccgccagcatgattaaacgctacgacgagcaccatcaggacctcacgctgctcaaggcactcgtccgccagcagctccccgagaagtacaaggagatcttcttcgaccaatcaaaaaacggctacgcgggatatatcgacggcggtgccagccaggaagagttctacaagttcatcaaaccaatcctggagaagatggacggcaccgaggagttgctggtcaagctcaacagggaggacctcctcaggaagcagaggaccttcgacaacggctccatcccgcatcagatccacctgggcgaactgcatgccatcctgcggcgccaggaggacttctacccgttcctgaaggataaccgggagaagatcgagaagatcttgacgttccgcatcccatactacgtgggcccgctggctcgcggcaactcccggttcgcctggatgacccggaagtcggaggagaccatcacaccctggaactttgaggaggtggtcgataagggcgctagcgctcagagcttcatcgagcgcatgaccaacttcgataaaaacctgcccaatgaaaaagtcctccccaagcactcgctgctctacgagtacttcaccgtgtacaacgagctcaccaaggtcaaatacgtcaccgagggcatgcggaagccggcgttcctgagcggcgagcagaagaaggcgatagtggacctcctcttcaagaccaacaggaaggtgaccgtgaagcaattaaaagaggactacttcaagaaaatagagtgcttcgactccgtggagatctcgggcgtggaggatcggttcaacgcctcactcggcacgtatcacgacctcctcaagatcattaaagacaaggacttcctcgacaacgaggagaacgaggacatcctcgaggacatcgtcctcaccctgaccctgttcgaggaccgcgaaatgatcgaggagaggctgaagacctacgcgcacctgttcgacgacaaggtcatgaaacagctcaagaggcgccgctacactggttggggaaggctgtcccgcaagctcattaatggcatcagggacaagcagagcggcaagaccatcctggacttcctcaagtccgacgggttcgccaaccgcaacttcatgcagctcattcacgacgactcgctcacgttcaaggaagacatccagaaggcacaggtgagcgggcagggtgactccctccacgaacacatcgccaacctggccggctcgccggccattaaaaagggcatcctgcagacggtcaaggtcgtcgacgagctcgtgaaggtgatgggccggcacaagcccgaaaatatcgtcatagagatggccagggagaaccagaccacccaaaaagggcagaagaactcgcgcgagcggatgaaacggatcgaggagggcattaaagagctcgggtcccagatcctgaaggagcaccccgtggaaaatacccagctccagaatgaaaagctctacctctactacctgcagaacggccgcgacatgtacgtggaccaggagctggacattaatcggctatcggactacgacgtcgaccacatcgtgccgcagtcgttcctcaaggacgatagcatcgacaacaaggtgctcacccggtcggataaaaatcggggcaagagcgacaacgtgcccagcgaggaggtcgtgaagaagatgaaaaactactggcgccagctcctcaacgcgaaactgatcacccagcgcaagttcgacaacctgacgaaggcggaacgcggtggcttgagcgaactcgataaggcgggcttcataaaaaggcagctggtcgagacgcgccagatcacgaagcatgtcgcccagatcctggacagccgcatgaatactaagtacgatgaaaacgacaagctgatccgggaggtgaaggtgatcacgctgaagtccaagctcgtgtcggacttccgcaaggacttccagttctacaaggtccgcgagatcaacaactaccaccacgcccacgacgcctacctgaatgcggtggtcgggaccgccctgatcaagaagtacccgaagctggagtcggagttcgtgtacggcgactacaaggtctacgacgtgcgcaaaatgatcgccaagtccgagcaggagatcggcaaggccacggcaaaatacttcttctactcgaacatcatgaacttcttcaagaccgagatcaccctcgcgaacggcgagatccgcaagcgcccgctcatcgaaaccaacggcgagacgggcgagatcgtctgggataagggccgggatttcgcgacggtccgcaaggtgctctccatgccgcaagtcaatatcgtgaaaaagacggaggtccagacgggcgggttcagcaaggagtccatcctcccgaagcgcaactccgacaagctcatcgcgaggaagaaggattgggacccgaaaaaatatggcggcttcgacagcccgaccgtcgcatacagcgtcctcgtcgtggcgaaggtggagaagggcaagtcaaagaagctcaagtccgtgaaggagctgctcgggatcacgattatggagcggtcctccttcgagaagaacccgatcgacttcctagaggccaagggatataaggaggtcaagaaggacctgattattaaactgccgaagtactcgctcttcgagctggaaaacggccgcaagaggatgctcgcctccgcaggcgagttgcagaagggcaacgagctcgccctcccgagcaaatacgtcaatttcctgtacctcgctagccactatgaaaagctcaagggcagcccggaggacaacgagcagaagcagctcttcgtggagcagcacaagcattacctggacgagatcatcgagcagatcagcgagttctcgaagcgggtgatcctcgccgacgcgaacctggacaaggtgctgtcggcatataacaagcaccgcgacaaaccaatacgcgagcaggccgaaaatatcatccacctcttcaccctcaccaacctcggcgctccggcagccttcaagtacttcgacaccacgattgaccggaagcggtacacgagcacgaaggaggtgctcgatgcgacgctgatccaccagagcatcacagggctctatgaaacacgcatcgacctgagccagctgggcggagac

SEQ ID NO: 45 - protein, 1368 aa, Artificial Sequence [sequence omitted]

SEQ ID NO: 46 - protein, 7 aa, SV40
PKKKRKV

SEQ ID NO: 47 - protein, 7 aa, T. reesei
KKKKLKL

SEQ ID NO: 48 - protein, 1388 aa, Streptococcus thermophilus
MTKPYSIGLDIGTNSVGWAVTTDNYKVPSKKMKVLGNTSKKYIKKNLLGVLLFDSGITAEGRRLKRTARRRYTRRRNRILYLQEIFSTEMATLDDAFFQRLDDSFLVPDDKRDSKYPIFGNLVEEKAYHDEFPTIYHLRKYLADSTKKADLRLVYLALAHMIKYRGHFLIEGEFNSKNNDIQKNFQDFLDTYNAIFESDLSLENSKQLEEIVKDKISKLEKKDRILKLFPGEKNSGIFSEFLKLIVGNQADFRKCFNLDEKASLHFSKESYDEDLETLLGYIGDDYSDVFLKAKKLYDAILLSGFLTVTDNETEAPLSSAMIKRYNEHKEDLALLKEYIRNISLKTYNEVFKDDTKNGYAGYIDGKTNQEDFYVYLKKLLAEFEGADYFLEKIDREDFLRKQRTFDNGSIPYQIHLQEMRAILDKQAKFYPFLAKNKERIEKILTFRIPYYVGPLARGNSDFAWSIRKRNEKITPWNFEDVIDKESSAEAFINRMTSFDLYLPEEKVLPKHSLLYETFNVYNELTKVRFIAESMRDYQFLDSKQKKDIVRLYFKDKRKVTDKDIIEYLHAIYGYDGIELKGIEKQFNSSLSTYHDLLNIINDKEFLDDSSNEAIIEEIIHTLTIFEDREMIKQRLSKFENIFDKSVLKKLSRRHYTGWGKLSAKLINGIRDEKSGNTILDYLIDDGISNRNFMQLIHDDALSFKKKIQKAQIIGDEDKGNIKEVVKSLPGSPAIKKGILQSIKIVDELVKVMGGRKPESIVVEMARENQYTNQGKSNSQQRLKRLEKSLKELGSKILKENIPAKLSKIDNNALQNDRLYLYYLQNGKDMYTGDDLDIDRLSNYDIDHIIPQAFLKDNSIDNKVLVSSASNRGKSDDVPSLEVVKKRKTFWYQLLKSKLISQRKFDNLTKAERGGLSPEDKAGFIQRQLVETRQITKHVARLLDEKFNNKKDENNRAVRTVKIITLKSTLVSQFRKDFELYKVREINDFHHAHDAYLNAVVASALLKKYPKLEPEFVYGDYPKYNSFRERKSATEKVYFYSNIMNIFKKSISLADGRVIERPLIEVNEETGESVWNKESDLATVRRVLSYPQVNVVKKVEEQNHGLDRGKPKGLFNANLSSKPKPNSNENLVGAKEYLDPKKYGGYAGISNSFTVLVKGTIEKGAKKKITNVLEFQGISILDRINYRKDKLNFLLEKGYKDIELIIELPKYSLFELSDGSRRMLASILSTNNKRGEIHKGNQIFLSQKFVKLLYHAKRISNTINENHRKYVENHKKEFEELFYYILEFNENYVGAKKNGKLLNSAFQSWQNHSIDELCSSFIGPTGSERKGLFELTSRGSAADFEFLGVKIPRYRDYTPSSLLKDATLIHQSVTGLYETRIDLAKLGEG

SEQ ID NO: 49 - protein, 1345 aa, Streptococcus mutans
MKKPYSIGLDIGTNSVGWAVVTDDYKVPAKKMKVLGNTDKSHIEKNLLGALLFDSGNTAEDRRLKRTARRRYTRRRNRILYLQEIFSEEMGKVDDSFFHRLEDSFLVTEDKRGERHPIFGNLEEEVKYHENFPTIYHLRQYLADNPEKVDLRLVYLALAHIIKFRGHFLIEGKFDTRNNDVQRLFQEFLAVYDNTFENSSLQEQNVQVEEILTDKISKSAKKDRVLKLFPNEKSNGRFAEFLKLIVGNQADFKKHFELEEKAPLQFSKDTYEEELEVLLAQIGDNYAELFLSAKKLYDSILLSGILTVTDVGTKAPLSASMIQRYNEHQMDLAQLKQFIRQKLSDKYNEVFSDVSKDGYAGYIDGKTNQEAFYKYLKGLLNKIEGSGYFLDKIEREDFLRKQRTFDNGSIPHQIHLQEMRAIIRRQAEFYPFLADNQDRIEKLLTFRIPYYVGPLARGKSDFAWLSRKSADKITPWNFDEIVDKESSAEAFINRMTNYDLYLPNQKVLPKHSLLYEKFTVYNELTKVKYKTEQGKTAFFDANMKQEIFDGVFKVYRKVTKDKLMDFLEKEFDEFRIVDLTGLDKENKVFNASYGTYHDLCKILDKDFLDNSKNEKILEDIVLTLTLFEDREMIRKRLENYSDLLTKEQVKKLERRHYTGWGRLSAELIHGIRNKESRKTILDYLIDDGNSNRNFMQLINDDALSFKEEIAKAQVIGETDNLNQVVSDIAGSPAIKKGILQSLKIVDELVKIMGHQPENIVVEMARENQFTNQGRRNSQQRLKGLTDSIKEFGSQILKEHPVENSQLQNDRLFLYYLQNGRDMYTGEELDIDYLSQYDIDHIIPQAFIKDNSIDNRVLTSSKENRGKSDDVPSKDVVRKMKSYWSKLLSAKLITQRKFDNLTKAERGGLTDDDKAGFIKRQLVETRQITKHVARILDERFNTETDENNKKIRQVKIVTLKSNLVSNFRKEFELYKVREINDYHHAHDAYLNAVIGKALLGVYPQLEPEFVYGDYPHFHGHKENKATAKKFFYSNIMNFFKKDDVRTDKNGEIIWKKDEHISNIKKVLSYPQVNIVKKVEEQTGGFSKESILPKGNSDKLIPRKTKKFYWDTKKYGGFDSPIVAYSILVIADIEKGKSKKLKTVKALVGVTIMEKMTFERDPVAFLERKGYRNVQEENIIKLPKYSLFKLENGRKRLLASARELQKGNEIVLPNHLGTLLYHAKNIHKVDEPKHLDYVDKHKDEFKELLDVVSNFSKKYTLAEGNLEKIKELYAQNNGEDLKELASSFINLLTFTAIGAPATFKFFDKNIDRKRYTSTTEILNATLIHQSITGLYETRIDLNKLGGD

SEQ ID NO: 50 - protein, 984 aa, Campylobacter jejuni
MARILAFDIGISSIGWAFSENDELKDCGVRIFTKVENPKTGESLALPRRLARSARKRLARRKARLNHLKHLIANEFKLNYEDYQSFDESLAKAYKGSLISPYELRFRALNELLSKQDFARVILHIAKRRGYDDIKNSDDKEKGAILKAIKQNEEKLANYQSVGEYLYKEYFQKFKENSKEFTNVRNKKESYERCIAQSFLKDELKLIFKKQREFGFSFSKKFEEEVLSVAFYKRALKDFSHLVGNCSFFTDEKRAPKNSPLAFMFVALTRIINLLNNLKNTEGILYTKDDLNALLNEVLKNGTLTYKQTKKLLGLSDDYEFKGEKGTYFIEFKKYKEFIKALGEHNLSQDDLNEIAKDITLIKDEIKLKKALAKYDLNQNQIDSLSKLEFKDHLNISFKALKLVTPLMLEGKKYDEACNELNLKVAINEDKKDFLPAFNETYYKDEVTNPVVLRAIKEYRKVLNALLKKYGKVHKINIELAREVGKNHSQRAKIEKEQNENYKAKKDAELECEKLGLKINSKNILKLRLFKEQKEFCAYSGEKIKISDLQDEKMLEIDHIYPYSRSFDDSYMNKVLVFTKQNQEKLNQTPFEAFGNDSAKWQKIEVLAKNLPTKKQKRILDKNYKDKEQKNFKDRNLNDTRYIARLVLNYTKDYLDFLPLSDDENTKLNDTQKGSKVHVEAKSGMLTSALRHTWGFSAKDRNNHLHHAIDAVIIAYANNSIVKAFSDFKKEQESNSAELYAKKISELDYKNKRKFFEPFSGFRQKVLDKIDEIFVSKPERKKPSGALHEETFRKEEEFYQSYGGKEGVLKALELGKIRKVNGKIVKNGDMFRVDIFKHKKTNKFYAVPIYTMDFALKVLPNKAVARSKKGEIKDWILMDENYEFCFSLYKDSLILIQTKDMQEPEFVYYNAFTSSTVSLIVSKHDNKFETLSKNQKILFKNANEKEVIAKSIGIQNLKVFEKYIVSALGEVTKAEFRQREDFKK

SEQ ID NO: 51 - protein, 1082 aa, Neisseria meningitides
MAAFKPNSINYILGLDIGIASVGWAMVEIDEEENPIRLIDLGVRVFERAEVPKTGDSLAMARRLARSVRRLTRRRAHRLLRTRRLLKREGVLQAANFDENGLIKSLPNTPWQLRAAALDRKLTPLEWSAVLLHLIKHRGYLSQRKNEGETADKELGALLKGVAGNAHALQTGDFRTPAELALNKFEKESGHIRNQRSDYSHTFSRKDLQAELILLFEKQKEFGNPHVSGGLKEGIETLLMTQRPALSGDAVQKMLGHCTFEPAEPKAAKNTYTAERFIWLTKLNNLRILEQGSERPLTDTERATLMDEPYRKSKLTYAQARKLLGLEDTAFFKGLRYGKDNAEASTLMEMKAYHAISRALEKEGLKDKKSPLNLSPELQDEIGTAFSLFKTDEDITGRLKDRIQPEILEALLKHISFDKFVQISLKALRRIVPLMEQGKRYDEACAEIYGDHYGKKNTEEKIYLPPIPADEIRNPVVLRALSQARKVINGVVRRYGSPARIHIETAREVGKSFKDRKEIEKRQEENRKDREKAAAKFREYFPNFVGEPKSKDILKLRLYEQQHGKCLYSGKEINLGRLNEKGYVEIDHALPFSRTWDDSFNNKVLVLGSENQNKGNQTPYEYFNGKDNSREWQEFKARVETSRFPRSKKQRILLQKFDEDGFKERNLNDTRYVNRFLCQFVADRMRLTGKGKKRVFASNGQITNLLRGFWGLRKVRAENDRHHALDAVVVACSTVAMQQKITRFVRYKEMNAFDGKTIDKETGEVLHQKTHFPQPWEFFAQEVMIRVFGKPDGKPEFEEADTLEKLRTLLAEKLSSRPEAVHEYVTPLFVSRAPNRKMSGQGHMETVKSAKRLDEGVSVLRVPLTQLKLKDLEKMVNREREPKLYEALKARLEAHKDDPAKAFAEPFYKYDKAGNRTQQVKAVRVEQVQKTGVWVRNHNGIADNATMVRVDVFEKGDKYYLVPIYSWQVAKGILPDRAVVQGKDEEDWQLIDDSFNFKFSLHPNDLVEVITKKARMFGYFASCHRGTGNINIRIHDLDHKIGKNGILEGIGVKTALSFQKYQIDELGKEIRPCRLKKRPPVR

SEQ ID NO: 52 - protein, 1629 aa, Francisella tularensis
MNFKILPIAIDLGVKNTGVFSAFYQKGTSLERLDNKNGKVYELSKDSYTLLMNNRTARRHQRRGIDRKQLVKRLFKLIWTEQLNLEWDKDTQQAISFLFNRRGFSFITDGYSPEYLNIVPEQVKAILMDIFDDYNGEDDLDSYLKLATEQESKISEIYNKLMQKILEFKLMKLCTDIKDDKVSTKTLKEITSYEFELLADYLANYSESLKTQKFSYTDKQGNLKELSYYHHDKYNIQEFLKRHATINDRILDTLLTDDLDIWNFNFEKFDFDKNEEKLQNQEDKDHIQAHLHHFVFAVNKIKSEMASGGRHRSQYFQEITNVLDENNHQEGYLKNFCENLHNKKYSNLSVKNLVNLIGNLSNLELKPLRKYFNDKIHAKADHWDEQKFTETYCHWILGEWRVGVKDQDKKDGAKYSYKDLCNELKQKVTKAGLVDFLLELDPCRTIPPYLDNNNRKPPKCQSLILNPKFLDNQYPNWQQYLQELKKLQSIQNYLDSFETDLKVLKSSKDQPYFVEYKSSNQQIASGQRDYKDLDARILQFIFDRVKASDELLLNEIYFQAKKLKQKASSELEKLESSKKLDEVIANSQLSQILKSQHTNGIFEQGTFLHLVCKYYKQRQRARDSRLYIMPEYRYDKKLHKYNNTGRFDDDNQLLTYCNHKPRQKRYQLLNDLAGVLQVSPNFLKDKIGSDDDLFISKWLVEHIRGFKKACEDSLKIQKDNRGLLNHKINIARNTKGKCEKEIFNLICKIEGSEDKKGNYKHGLAYELGVLLFGEPNEASKPEFDRKIKKFNSIYSFAQIQQIAFAERKGNANTCAVCSADNAHRMQQIKITEPVEDNKDKIILSAKAQRLPAIPTRIVDGAVKKMATILAKNIVDDNWQNIKQVLSAKHQLHIPIITESNAFEFEPALADVKGKSLKDRRKKALERISPENIFKDKNNRIKEFAKGISAYSGANLTDGDFDGAKEELDHIIPRSHKKYGTLNDEANLICVTRGDNKNKGNRIFCLRDLADNYKLKQFETTDDLEIEKKIADTIWDANKKDFKFGNYRSFINLTPQEQKAFRHALFLADENPIKQAVIRAINNRNRTFVNGTQRYFAEVLANNIYLRAKKENLNTDKISFDYFGIPTIGNGRGIAEIRQLYEKVDSDIQAYAKGDKPQASYSHLIDAMLAFCIAADEHRNDGSIGLEIDKNYSLYPLDKNTGEVFTKDIFSQIKITDNEFSDKKLVRKKAIEGFNTHRQMTRDGIYAENYLPILIHKELNEVRKGYTWKNSEEIKIFKGKKYDIQQLNNLVYCLKFVDKPISIDIQISTLEELRNILTTNNIAATAEYYYINLKTQKLHEYYIENYNTALGYKKYSKEMEFLRSLAYRSERVKIKSIDDVKQVLDKDSNFIIGKITLPFKKEWQRLYREWQNTTIKDDYEFLKSFFNVKSITKLHKKVRKDFSLPISTNEGKFLVKRKTWDNNFIYQILNDSDSRADGTKPFIPAFDISKNEIVEAIIDSFTSKNIFWLPKNIELQKVDNKNIFAIDTSKWFEVETPSDLRDIGIATIQYKIDNNSRPKVRVKLDYVIDDDSKINYFMNHSLLKSRYPDKVLEILKQSTIIEFESSGFNKTIKEMLGMKLAGIYNETSNN

SEQ ID NO: 53 - protein, 1056 aa, Pasteurella multocida
MQTTNLSYILGLDLGIASVGWAVVEINENEDPIGLIDVGVRIFERAEVPKTGESLALSRRLARSTRRLIRRRAHRLLLAKRFLKREGILSTIDLEKGLPNQAWELRVAGLERRLSAIEWGAVLLHLIKHRGYLSKRKNESQTNNKELGALLSGVAQNHQLLQSDDYRTPAELALKKFAKEEGHIRNQRGAYTHTFNRLDLLAELNLLFAQQHQFGNPHCKEHIQQYMTELLMWQKPALSGEAILKMLGKCTHEKNEFKAAKHTYSAERFVWLTKLNNLRILEDGAERALNEEERQLLINHPYEKSKLTYAQVRKLLGLSEQAIFKHLRYSKENAESATFMELKAWHAIRKALENQGLKDTWQDLAKKPDLLDEIGTAFSLYKTDEDIQQYLTNKVPNSVINALLVSLNFDKFIELSLKSLRKILPLMEQGKRYDQACREIYGHHYGEANQKTSQLLPAIPAQEIRNPVVLRTLSQARKVINAIIRQYGSPARVHIETGRELGKSFKERREIQKQQEDNRTKRESAVQKFKELFSDFSSEPKSKDILKFRLYEQQHGKCLYSGKEINIHRLNEKGYVEIDHALPFSRTWDDSFNNKVLVLASENQNKGNQTPYEWLQGKINSERWKNFVALVLGSQCSAAKKQRLLTQVIDDNKFIDRNLNDTRYIARFLSNYIQENLLLVGKNKKNVFTPNGQITALLRSRWGLIKARENNNRHHALDAIVVACATPSMQQKITRFIRFKEVHPYKIENRYEMVDQESGEIISPHFPEPWAYFRQEVNIRVFDNHPDTVLKEMLPDRPQANHQFVQPLFVSRAPTRKMSGQGHMETIKSAKRLAEGISVLRIPLTQLKPNLLENMVNKEREPALYAGLKARLAEFNQDPAKAFATPFYKQGGQQVKAIRVEQVQKSGVLVRENNGVADNASIVRTDVFIKNNKFFLVPIYTWQVAKGILPNKAIVAHKNEDEWEEMDEGAKFKFSLFPNDLVELKTKKEYFFGYYIGLDRATGNISLKEHDGEISKGKDGVYRVGVKLALSFEKYQVDELGKNRQICRPQQRQPVR

SEQ ID NO: 54 - DNA, 4284 bp, Artificial Sequence
  Synthetic construct
atgcaccatcatcatcatcattcttctggtctggtgccacgcggttctggtatgaaagaaaccgctgctgctaaattcgaacgccagcacatggacagcccagatctgggtaccgacgacgacgacaaggccatggccccaaaaaagaaacgcaaggttatggataaaaaatacagcattggtctggccatcggaaccaacagcgttgggtgggcagtaataacagatgaatacaaagtgccgtcaaaaaaatttaaggttctggggaatacagatcgccacagcataaaaaagaatctgattggggcattgctgtttgattcgggtgagacagctgaggccacgcgtctgaaacgtacagcaagaagacgttacacacgtcgtaaaaatcgtatttgctacttacaggaaattttttctaacgaaatggccaaggtagatgatagtttcttccatcgtctcgaagaatcttttctggttgaggaagataaaaaacacgaacgtcaccctatctttggcaatatcgtggatgaagtggcctatcatgaaaaataccctacgatttatcatcttcgcaagaagttggttgatagtacggacaaagcggatctgcgtttaatctatcttgcgttagcgcacatgatcaaatttcgtggtcatttcttaattgaaggtgatctgaatcctgataactctgatgtggacaaattgtttatacaattagtgcaaacctataatcagctgttcgaggaaaaccccattaatgcctctggagttgatgccaaagcgattttaagcgcgagactttctaagtcccggcgtctggagaatctgatcgcccagttaccaggggaaaagaaaaatggtctgtttggtaatctgattgccctcagtctggggcttaccccgaacttcaaatccaattttgacctggctgaggacgcaaagctgcagctgagcaaagatacttatgatgatgacctcgacaatctgctcgcccagattggtgaccaatatgcggatctgtttctggcagcgaagaatctttcggatgctatcttgctgtcggatattctgcgtgttaataccgaaatcaccaaagcgcctctgtctgcaagtatgatcaagagatacgacgagcaccaccaggacctgactcttcttaaggcactggtacgccaacagcttccggagaaatacaaagaaatattcttcgaccagtccaagaatggttacgcgggctacatcgatggtggtgcatcacaggaagagttctataaatttattaaaccaatccttgagaaaatggatggcacggaagagttacttgttaaacttaaccgcgaagacttgcttagaaagcaacgtacattcgacaacggctccatcccacaccagattcatttaggtgaacttcacgccatcttgcgcagacaagaagatttctatcccttcttaaaagacaatcgggagaaaatcgagaagatcctgacgttccgcattccctattatgtcggtcccctggcacgtggtaattctcggtttgcctggatgacgcgcaaaagtgaggaaaccatcaccccttggaactttgaagaagtcgtggataaaggtgctagcgcgcagtcttttatagaaagaatgacgaacttcgataaaaacttgcccaacgaaaaagtcctgcccaagcactctcttttatatgagtactttactgtgtacaacgaactgactaaagtgaaatacgttacggaaggtatgcgcaaacctgcctttcttagtggcgagcagaaaaaagcaattgtcgatcttctctttaaaacgaatcgcaaggtaactgtaaaacagctgaaggaagattatttcaaaaagatcgaatgctttgattctgtcgagatctcgggtgtcgaagatcgtttcaacgcttccttagggacctatcatgatttgctgaagataataaaagacaaagactttctcgacaatgaagaaaatgaagatattctggaggatattgttttgaccttgaccttattcgaagatagagagatgatcgaggagcgcttaaaaacctatgcccacctgtttgatgacaaagtcatgaagcaattaaagcgccgcagatatacggggtggggccgcttgagccgcaagttgattaacggtattagagacaagcagagcggaaaaactatcctggatttcctcaaatctgacggatttgcgaaccgcaattttatgcagcttatacatgatgattcgcttacattcaaagaggatattcagaaggctcaggtgtctgggcaaggtgattcactccacgaacatatagcaaatttggccggctctcctgcgattaagaaggggatcctgcaaacagttaaagttgtggatgaacttgtaaaagtaatgggccgccacaagccggagaatatcgtgatagaaatggcgcgcgagaatcaaacgacacaaaaaggtcaaaagaactcaagagagagaatgaagcgcattgaggaggggataaaggaacttggatctcaaattctgaaagaacatccagttgaaaacactcagctgcaaaatgaaaaattgtacctgtactacctgcagaatggaagagacatgtacgtggatcaggaattggatatcaatagactctcggactatgacgtagatcacattgtccctcagagcttcctcaaggatgattctatagataataaagtacttacgagatcggacaaaaatcgcggtaaatcggataacgtcccatcggaggaagtcgttaaaaagatgaaaaactattggcgtcaactgctgaacgccaagctgatcacacagcgtaagtttgataatctgactaaagccgaacgcggtggtcttagtgaactcgataaagcaggatttataaaacggcagttagtagaaacgcgccaaattacgaaacacgtggctcagatcctcgattctagaatgaatacaaagtacgatgaaaacgataaactgatccgtgaagtaaaagtcattaccttaaaatctaaacttgtgtccgatttccgcaaagattttcagttttacaaggtccgggaaatcaataactatcaccatgcacatgatgcatatttaaatgcggttgtaggcacggcccttattaagaaataccctaaactcgaaagtgagtttgtttatggggattataaagtgtatgacgttcgcaaaatgatcgcgaaatcagaacaggaaatcggtaaggctaccgctaaatactttttttattccaacattatgaatttttttaagaccgaaataactctcgcgaatggtgaaatccgtaaacggcctcttatagaaaccaatggtgaaacgggagaaatcgtttgggataaaggtcgtgactttgccaccgttcgtaaagtcctctcaatgccgcaagttaacattgtcaagaagacggaagttcaaacagggggattctccaaagaatctatcctgccgaagcgtaacagtgataaacttattgccagaaaaaaagattgggatccaaaaaaatacggaggctttgattcccctaccgtcgcgtatagtgtgctggtggttgctaaagtcgagaaagggaaaagcaagaaattgaaatcagttaaagaactgctgggtattacaattatggaaagatcgtcctttgagaaaaatccgatcgactttttagaggccaaggggtataaggaagtgaaaaaagatctcatcatcaaattaccgaagtatagtctttttgagctggaaaacggcagaaaaagaatgctggcctccgcgggcgagttacagaagggaaatgagctggcgctgccttccaaatatgttaattttctgtaccttgccagtcattatgagaaactgaagggcagccccgaagataacgaacagaaacaattattcgtggaacagcataagcactatttagatgaaattatagagcaaattagtgaattttctaagcgcgttatcctcgcggatgctaatttagacaaagtactgtcagcttataataaacatcgggataagccgattagagaacaggccgaaaatatcattcatttgtttaccttaaccaaccttggagcaccagctgccttcaaatatttcgataccacaattgatcgtaaacggtatacaagtacaaaagaagtcttggacgcaaccctcattcatcaatctattactggattatatgagacacgcattgatctttcacagctgggcggagacaagaagaaaaaactgaaactg

SEQ ID NO: 55 - protein, 1428 aa, Artificial Sequence
  protein expressed from synthetic construct
MHHHHHHSSGLVPRGSGMKETAAAKFERQHMDSPDLGTDDDDKAMAPKKKRKVMDKKYSIGLAIGTNSVGWAVITDEYKVPSKKFKVLGNTDRHSIKKNLIGALLFDSGETAEATRLKRTARRRYTRRKNRICYLQEIFSNEMAKVDDSFFHRLEESFLVEEDKKHERHPIFGNIVDEVAYHEKYPTIYHLRKKLVDSTDKADLRLIYLALAHMIKFRGHFLIEGDLNPDNSDVDKLFIQLVQTYNQLFEENPINASGVDAKAILSARLSKSRRLENLIAQLPGEKKNGLFGNLIALSLGLTPNFKSNFDLAEDAKLQLSKDTYDDDLDNLLAQIGDQYADLFLAAKNLSDAILLSDILRVNTEITKAPLSASMIKRYDEHHQDLTLLKALVRQQLPEKYKEIFFDQSKNGYAGYIDGGASQEEFYKFIKPILEKMDGTEELLVKLNREDLLRKQRTFDNGSIPHQIHLGELHAILRRQEDFYPFLKDNREKIEKILTFRIPYYVGPLARGNSRFAWMTRKSEETITPWNFEEVVDKGASAQSFIERMTNFDKNLPNEKVLPKHSLLYEYFTVYNELTKVKYVTEGMRKPAFLSGEQKKAIVDLLFKTNRKVTVKQLKEDYFKKIECFDSVEISGVEDRFNASLGTYHDLLKIIKDKDFLDNEENEDILEDIVLTLTLFEDREMIEERLKTYAHLFDDKVMKQLKRRRYTGWGRLSRKLINGIRDKQSGKTILDFLKSDGFANRNFMQLIHDDSLTFKEDIQKAQVSGQGDSLHEHIANLAGSPAIKKGILQTVKVVDELVKVMGRHKPENIVIEMARENQTTQKGQKNSRERMKRIEEGIKELGSQILKEHPVENTQLQNEKLYLYYLQNGRDMYVDQELDINRLSDYDVDHIVPQSFLKDDSIDNKVLTRSDKNRGKSDNVPSEEVVKKMKNYWRQLLNAKLITQRKFDNLTKAERGGLSELDKAGFIKRQLVETRQITKHVAQILDSRMNTKYDENDKLIREVKVITLKSKLVSDFRKDFQFYKVREINNYHHAHDAYLNAVVGTALIKKYPKLESEFVYGDYKVYDVRKMIAKSEQEIGKATAKYFFYSNIMNFFKTEITLANGEIRKRPLIETNGETGEIVWDKGRDFATVRKVLSMPQVNIVKKTEVQTGGFSKESILPKRNSDKLIARKKDWDPKKYGGFDSPTVAYSVLVVAKVEKGKSKKLKSVKELLGITIMERSSFEKNPIDFLEAKGYKEVKKDLIIKLPKYSLFELENGRKRMLASAGELQKGNELALPSKYVNFLYLASHYEKLKGSPEDNEQKQLFVEQHKHYLDEIIEQISEFSKRVILADANLDKVLSAYNKHRDKPIREQAENIIHLFTLTNLGAPAAFKYFDTTIDRKRYTSTKEVLDATLIHQSITGLYETRIDLSQLGGDKKKKLKL

SEQ ID NO: 56 - DNA, 4889 bp, Artificial Sequence
  Synthetic sequence
gactgtctccaccatgtaatttttccctgcgactccatataacgccggatcgtgaaattttcttctttcttttccttccttctcaacaaacaacggatctgtgctttgcggtcccctgcgttcacgcgtcagggtcgactgctctgcagctcgataactccatggagccatcaacttgctatggtgtcaatcatcctatcgacaggtccaagaacaagccggcctccggctgcctcattcgctgtcgcaagacggcttgagtgttgtggctggaggattcgggggccccatattccaacccttttttccaaggccgtcggccggtgaggttgaggaaaaccatgggttgcctacatattatcgatgctggtgtttggtagtagcaatgtttgcggtggcagtttgagccgagcctcgtcttgggcttctgacccaggcaacgccatctgactagctgcgccgaaggaaggatgattcattgtacgacgccagtcaatggaatcttcaagtaaaagcccgacgaaccgaccatgtcagatatcagaattctcctggctggtggggttggttggagactgcttacggagtcgatgcctcgtgactgtcatggccgcgtccagcctcctgggactctgtccgatattatgacacgagtaaagcctgcatgatgtcagtttgctgcgtctcatgtcgagaacaacacacctggtgctacataggcaatactacctcgtagcttcaaagttgactgttttgctttgatgtctttgatcatgcccatccatcccttgtcttgcagtgcatgtggatctctacgtccagacggggagaaagcttgtctgtgataaagtacgatgatgcattgatgcctgtggctacggcccttttatccccatcgtcatgcatctctatattaatccaggagactctcctcctggcatgggtgagtacaagtgacgaggacatgtagaagcagagccacgcaacgtcttgacatctgtacctattttgggccaaaaatcgagacccaccagctcgtcctaccttacatgtgaagatcttagcccacaatcctactgttttactagtattactgcacagctgtcatcacgagtcctcggttgcttgtgaaacccagctcagctcctgagcacatgcagtaacgccgactcggcgtcatttcgccacacccaatttggacctgagggatgctggaagctgctgagcagatcccgttaccgattcatggcactactacatccatacgcagcaaacatgggcttgggcttggcttctcaatgcaaaattgcccgcaaaagtcccggcattgtcgatgcagagatgcagatttcagcgggcgattctagggtagggcgactactactactaataccacctagtcagtatgtatctagcaccggaggctaggcggttagtggacgggaacctggtcattccatcgcaaccaggatcccgcacttcgttgcgcttctgcccccacggggcgggagttggcagaggcagaatgcggagcagccccttgtctgccctggccggggcctgttgaagcaagcagacgagagcagagcggttgagaagcggtggttgacgcttgacggtacgaagacgagcgagaatcccgttaagccgaggctgggctcccccccccgtcatcatcatgcccatcctgctcttccagcccactcgtctccctgcctcgtcgcctcccctccctcccccgattagctgcgcatgttctcctgacagcgtgactaatgacgcgttgccagcccattcgcctgacgcatcccggcatctgagtctagctcgtcacgctggcaatcttggcccaggcagagcagcaagacggcgggcatgattgggccgtgccctggcgggcatcagctggccatccgctgccacccgagaccgcatcaccgacttgtcggatctctccgagcagcaggaggctgatcctggccggcgagacgattgaaaagggctgccgggcccggagcaggacagcggcgagagcgagcgagagagaggaaaagaagaaggtcgactgtcttattttcagccagccccggctcaacagaagcagaggagaaggcgaacgacgtcaacgacgacgacgacgacgacgaagacggtgaagtccgttagttgaagatccttgccgtcacaacaccatctcgtggatattgctttcccctgccgttgcgttgccacctgttccctctttctcttccccccttcttcctcattccgagcgctactggttcctactccgcagccttcggttgtgcctttctctttgtcgaccattgcaccgcccgtcgcggcacttgggccccggagaattcggccctttcgcagcattttggccctcagttccccatggggacggtccacacttcctctcttggccctgcagaccttttgtcgtcggtccgagtcggaagaagctcagtcttgagcgcttgagtagcatctacgcgcgaatcactggacaaagtcggcaagacgaagccgtcgtcgcctgctgctgctgctgttactgcgacaggcgctccgactgggggcatcggcataataaaaagatgcccgccttcgccatggacctggccatgagccactcggcatcggctctctctctcaacgcttcctctcacacatcctccttcattccgcccatcatgcacgtcctgtcgactgcggtgctgctcggctccgttgccgttcaaaaggtcctgggaagaccaggatcaagcggtctgtccgacgtcaccaagaggtctgttgacgacttcatcagcaccgagacgcctattgcactgaacaatcttctttgcaatgttggtcctgatggatgccgtgcattcggcacatcagctggtgcggtgattgcatctcccagcacaattgacccggactgtaagttggccttgatgaaccatatcatatatcgccgagaagtggaccgcgtgctgagactgagacagactattacatgtggacgcgagatagcgctcttgtcttcaagaacctcatcgaccgcttcaccgaaacgtacgatgcgggcctgcagcgccgcatcgagcagtacattactgcccaggtcactctccagggcctctctaacccctcgggctccctcgcggacggctctggtctcggcgagcccaagtttgagttgaccctgaagcctttcaccggcaactggggtcgaccgcagcgggatggcccagctctgcgagccattgccttgattggatactcaaagtggctcatcaacaacaactatcagtcgactgtgtccaacgtcatctggcctattgtgcgcaacgacctcaactatgttgcccagtactggtcagtgcttgcttgctcttgaattacgtctttgcttgtgtgtctaatgcctccaccacaggaaccaaaccggctttgacctctgggaagaagtcaatgggagctcattctttactgttgccaaccagcaccgaggtatgaagcaaatcctcgacattcgctgctactgcacatgagcattgttactgaccagctctacagcacttgtcgagggcgccactcttgctgccactcttggccagtcgggaagcgcttattcatctgttgctccccaggttttgtgctttctccaacgattctgggtgtcgtctggtggatacgtcgactccaacagtatgtcttttcactgtttatatgagattggccaatactgatagctcgcctctagtcaacaccaacgagggcaggactggcaaggatgtcaactccgtcctgacttccatccacaccttcgatcccaaccttggctgtgacgcaggcaccttccagccatgcagtgacaaagcgctctccaacctcaaggttgttgtcgactccttccgctccatctacggcgtgaacaagggcattcctgccggtgctgccgtcgccattggccggtatgcagaggatgtgtactacaacggcaacccttggtatcttgctacatttgctgctgccgagcagctgtacgatgccatctacgtctggaagaagacgggctccatcacggtgaccgccacctccctggccttcttccaggagcttgttcctggcgtgacggccgggacctactccagcagctcttcgacctttaccaacatcatcaacgccgtctcgacatacgccgatggcttcctcagcgaggctgccaagtacgtccccgccgacggttcgctggccgagcagtttgaccgcaacagcggcactccgctgtctgcgcttcacctgacgtggtcgtacgcctcgttcttgacagccacggcccgtcgggctggcatcgtgcccccctcgtgggccaacagcagcgctagcacgatcccctcgacgtgctccggcgcgtccgtggtcggatcctactcgcgtcccaccgccacgtcattccctccgtcgcagacgcccaagcctggcgtgccttccggtactccctacacgcccctgccctgcgcgaccccaacctccgtggccgtcaccttccacgagctcgtgtcgacacagtttggccagacggtcaaggtggcgggcaacgccgcggccctgggcaactggagcacgagcgccgccgtggctctggacgccgtcaactatgccgataaccaccccctgtggattgggacggtcaacctcgaggctggagacgtcgtggagtacaagtacatcaatgtgggccaagatggctccgtgacctgggagagtgatcccaaccacacttacacggttcctgcggtggcttgtgtgacgcaggttgtcaaggaggacacctggcagtcgtaatgaatcggcaaggggtagtactagtagacttgtagtctgcc

SEQ ID NO: 57 - DNA, 25 bp, Artificial Sequence
  Primer
gactgtctccaccatgtaatttttc

SEQ ID NO: 58 - DNA, 27 bp, Artificial Sequence
  Primer
ggcagactacaagtctactagtactac

SEQ ID NO: 59 - DNA, 111 bp, Artificial Sequence
  Synthetic sequence
taatacgactcactatagggaagaccaggatcaaggttttagagctagaaatagcaagttaaaataaggctagtccgttatcaacttgaaaaagtggcaccgagtcggtgc

SEQ ID NO: 60 - DNA, 111 bp, Artificial Sequence
  Synthetic sequence
taatacgactcactataggacagaccgcttgatccgttttagagctagaaatagcaagttaaaataaggctagtccgttatcaacttgaaaaagtggcaccgagtcggtgc

SEQ ID NO: 61 - DNA, 4248 bp, Artificial Sequence
  Synthetic sequence
ccctgcctcgtcgcctcccctccctcccccgattagctgcgcatgttctcctgacagcgtgactaatgacgcgttgccagcccattcgcctgacgcatcccggcatctgagtctagctcgtcacgctggcaatcttggcccaggcagagcagcaagacggcgggcatgattgggccgtgccctggcgggcatcagctggccatccgctgccacccgagaccgcatcaccgacttgtcggatctctccgagcagcaggaggctgatcctggccggcgagacgattgaaaagggctgccgggcccggagcaggacagcggcgagagcgagcgagagagaggaaaagaagaaggtcgactgtcttattttcagccagccccggctcaacagaagcagaggagaaggcgaacgacgtcaacgacgacgacgacgacgacgaagacggtgaagtccgttagttgaagatccttgccgtcacaacaccatctcgtggatattgctttcccctgccgttgcgttgccacctgttccctctttctcttccccccttcttcctcattccgagcgctactggttcctactccgcagccttcggttgtgcctttctctttgtcgaccattgcaccgcccgtcgcggcacttgggccccggagaattcggccctttcgcagcattttggccctcagttccccatggggacggtccacacttcctctcttggccctgcagaccttttgtcgtcggtccgagtcggaagaagctcagtcttgagcgcttgagtagcatctacgcgcgaatcactggacaaagtcggcaagacgaagccgtcgtcgcctgctgctgctgctgttactgcgacaggcgctccgactgggggcatcggcataataaaaagatgcccgccttcgccatggacctggccatgagccactcggcatcggctctctctctcaacgcttcctctcacacatcctccttcattccgcccatcatggtttaaacctcgagtttataagtgacaacatgctctcaaagcgctcatggctggcacaagcctggaaagaaccaacacaaagcatactgcagcaaatcagctgaattcgtcaccaattaagtgaacatcaacctgaaggcagagtatgaggccagaagcacatctggatcgcagatcatggattgcccctcttgttgaagatgagaatctagaaagatggcggggtatgagataagagcgatgggggggcacatcatcttccaagacaaacaacctttgcagagtcaggcaatttttcgtataagagcaggaggagggagtccagtcatttcatcagcggtaaaatcactctagacaatcttcaagatgagttctgccttgggtgacttatagccatcatcatacctagacagaagcttgtgggatactaagaccaacgtacaagctcgcactgtacgctttgacttccatgtgaaaactcgatacggcgcgcctctaaattttatagctcaaccactccaatccaacctctgcatccctctcactcgtcctgatctactgttcaaatcagagaataaggacactatccaaatccaacagaatggctaccacctcccagctgcctgcctacaagcaggacttcctcaaatccgccatcgacggcggcgtcctcaagtttggcagcttcgagctcaagtccaagcggatatccccctacttcttcaacgcgggcgaattccacacggcgcgcctcgccggcgccatcgcctccgcctttgcaaagaccatcatcgaggcccaggagaaggccggcctagagttcgacatcgtcttcggcccggcctacaagggcatcccgctgtgctccgccatcaccatcaagctcggcgagctggcgccccagaacctggaccgcgtctcctactcgtttgaccgcaaggaggccaaggaccacggcgagggcggcaacatcgtcggcgcttcgctcaagggcaagagggtcctgattgtcgacgacgtcatcaccgccggcaccgccaagagggacgccattgagaagatcaccaaggagggcggcatcgtcgccggcatcgtcgtggccctggaccgcatggagaagctccccgctgcggatggcgacgactccaagcctggaccgagtgccattggcgagctgaggaaggagtacggcatccccatctttgccatcctcactctggatgacattatcgatggcatgaagggctttgctacccctgaggatatcaagaacacggaggattaccgtgccaagtacaaggcgactgactgattgaggcgttcaatgtcagaagggagagaaagactgaaaaggtggaaagaagaggcaaattgttgttattattattattctatctcgaatcttctagatcttgtcgtaaataaacaagcgtaactagctagcctccgtacaactgcttgaatttgatacccgtatggagggcagttattttattttgtttttcaagattttccattcgccgttgaactcgtctcacatcgcgtgtattgcccggttgcccatgtgttctcctactaccccaagtccctcacgggttgtctcactttctttctcctttatcctccctattttttttcaagtcagcgacagagcagtcatatggggatacgtgcaactgggactcacaacaggccatcttatggcctaatagccggcgttggatccactagtcaattggtttaaacagcacatgcagtaacgccgactcggcgtcatttcgccacacccaatttggacctgagggatgctggaagctgctgagcagatcccgttaccgattcatggcactactacatccatacgcagcaaacatgggcttgggcttggcttctcaatgcaaaattgcccgcaaaagtcccggcattgtcgatgcagagatgcagatttcagcgggcgattctagggtagggcgactactactactaataccacctagtcagtatgtatctagcaccggaggctaggcggttagtggacgggaacctggtcattccatcgcaaccaggatcccgcacttcgttgcgcttctgcccccacggggcgggagttggcagaggcagaatgcggagcagccccttgtctgccctggccggggcctgttgaagcaagcagacgagagcagagcggttgagaagcggtggttgacgcttgacggtacgaagacgagcgagaatcccgttaagccgaggctgggctaattaattaatgaatcggcaaggggtagtactagtagacttgtagtctgccggattattgattggagttggtcagtagaatgaaccacgggaatattcggtcaccgggacatttgggatatagcgtttcgagaagctgctggttgcagcacattggagaaggatgcccttttacgacttataccgctatgccgggtatattaatttagccgttatgaaactcaaagagacgatgataatgatgacgagtaattgttcgtttcaatttcgaaagctgactcccacgaagaatatgccaatgacccacggcatgaagcctgaactgggcgtgtgtaacactttaatttgcctgacggcggacaaaacaaaggcggcagcaatgttgagaccgtgtgataaaccaaggttcccgagggagagagagagagagagagagagagagctaggtgaaagaatgagtccgcctttgagtcatcctgcgtctctctctccccctctctcactctctgtatcccatcaacctcttccctgttccttctcctatcgcatccatgcgtttgcatcttccatttcattctttccccttgagccccatctatgcaaactcatcatccggcgcctcgatggaatccttgaccttgatgagaatcgccgtcatccaaggctccagcctgctcgtgcggtcgaactggaacagcagctcgctaaactcatcctggctgtggttgtcgacggcgttgcacaggtcctcgagcagcttgtacttgtattgagaggagaactcggggtccttttggcggtaggactcgacggcgcggcgggtgccgaccatgtcgcccgtggcgaggtggcagatgccggccttgaagcagtaggtcgagaggctccacttcatggtgccgttgccgatcatggtgttgatgatgcggtcgtacgtctcgatggcgccgtagtagtcgccgtcgagggcggcgaggtcggcgtactgcgtccagagctt

SEQ ID NO: 62 - DNA, 30 bp, Artificial Sequence
  Primer
cactactacatccatacgcagcaaacatgg

SEQ ID NO: 63 - DNA, 26 bp, Artificial Sequence
  Primer
ggtcaagaagcacatgccagagttcg

SEQ ID NO: 64 - DNA, 25 bp, Artificial Sequence
  Primer
gactgtctccaccatgtaatttttc

SEQ ID NO: 65 - DNA, 4104 bp, Artificial Sequence
  codon optimized seqs
atggataaaaaatacagcattggtctggccatcggaaccaacagcgttgggtgggcagtaataacagatgaatacaaagtgccgtcaaaaaaatttaaggttctggggaatacagatcgccacagcataaaaaagaatctgattggggcattgctgtttgattcgggtgagacagctgaggccacgcgtctgaaacgtacagcaagaagacgttacacacgtcgtaaaaatcgtatttgctacttacaggaaattttttctaacgaaatggccaaggtagatgatagtttcttccatcgtctcgaagaatcttttctggttgaggaagataaaaaacacgaacgtcaccctatctttggcaatatcgtggatgaagtggcctatcatgaaaaataccctacgatttatcatcttcgcaagaagttggttgatagtacggacaaagcggatctgcgtttaatctatcttgcgttagcgcacatgatcaaatttcgtggtcatttcttaattgaaggtgatctgaatcctgataactctgatgtggacaaattgtttatacaattagtgcaaacctataatcagctgttcgaggaaaaccccattaatgcctctggagttgatgccaaagcgattttaagcgcgagactttctaagtcccggcgtctggagaatctgatcgcccagttaccaggggaaaagaaaaatggtctgtttggtaatctgattgccctcagtctggggcttaccccgaacttcaaatccaattttgacctggctgaggacgcaaagctgcagctgagcaaagatacttatgatgatgacctcgacaatctgctcgcccagattggtgaccaatatgcggatctgtttctggcagcgaagaatctttcggatgctatcttgctgtcggatattctgcgtgttaataccgaaatcaccaaagcgcctctgtctgcaagtatgatcaagagatacgacgagcaccaccaggacctgactcttcttaaggcactggtacgccaacagcttccggagaaatacaaagaaatattcttcgaccagtccaagaatggttacgcgggctacatcgatggtggtgcatcacaggaagagttctataaatttattaaaccaatccttgagaaaatggatggcacggaagagttacttgttaaacttaaccgcgaagacttgcttagaaagcaacgtacattcgacaacggctccatcccacaccagattcatttaggtgaacttcacgccatcttgcgcagacaagaagatttctatcccttcttaaaagacaatcgggagaaaatcgagaagatcctgacgttccgcattccctattatgtcggtcccctggcacgtggtaattctcggtttgcctggatgacgcgcaaaagtgaggaaaccatcaccccttggaactttgaagaagtcgtggataaaggtgctagcgcgcagtcttttatagaaagaatgacgaacttcgataaaaacttgcccaacgaaaaagtcctgcccaagcactctcttttatatgagtactttactgtgtacaacgaactgactaaagtgaaatacgttacggaaggtatgcgcaaacctgcctttcttagtggcgagcagaaaaaagcaattgtcgatcttctctttaaaacgaatcgcaaggtaactgtaaaacagctgaaggaagattatttcaaaaagatcgaatgctttgattctgtcgagatctcgggtgtcgaagatcgtttcaacgcttccttagggacctatcatgatttgctgaagataataaaagacaaagactttctcgacaatgaagaaaatgaagatattctggaggatattgttttgaccttgaccttattcgaagatagagagatgatcgaggagcgcttaaaaacctatgcccacctgtttgatgacaaagtcatgaagcaattaaagcgccgcagatatacggggtggggccgcttgagccgcaagttgattaacggtattagagacaagcagagcggaaaaactatcctggatttcctcaaatctgacggatttgcgaaccgcaattttatgcagcttatacatgatgattcgcttacattcaaagaggatattcagaaggctcaggtgtctgggcaaggtgattcactccacgaacatatagcaaatttggccggctctcctgcgattaagaaggggatcctgcaaacagttaaagttgtggatgaacttgtaaaagtaatgggccgccacaagccggagaatatcgtgatagaaatggcgcgcgagaatcaaacgacacaaaaaggtcaaaagaactcaagagagagaatgaagcgcattgaggaggggataaaggaacttggatctcaaattctgaaagaacatccagttgaaaacactcagctgcaaaatgaaaaattgtacctgtactacctgcagaatggaagagacatgtacgtggatcaggaattggatatcaatagactctcggactatgacgtagatcacattgtccctcagagcttcctcaaggatgattctatagataataaagtacttacgagatcggacaaaaatcgcggtaaatcggataacgtcccatcggaggaagtcgttaaaaagatgaaaaactattggcgtcaactgctgaacgccaagctgatcacacagcgtaagtttgataatctgactaaagccgaacgcggtggtcttagtgaactcgataaagcaggatttataaaacggcagttagtagaaacgcgccaaattacgaaacacgtggctcagatcctcgattctagaatgaatacaaagtacgatgaaaacgataaactgatccgtgaagtaaaagtcattaccttaaaatctaaacttgtgtccgatttccgcaaagattttcagttttacaaggtccgggaaatcaataactatcaccatgcacatgatgcatatttaaatgcggttgtaggcacggcccttattaagaaataccctaaactcgaaagtgagtttgtttatggggattataaagtgtatgacgttcgcaaaatgatcgcgaaatcagaacaggaaatcggtaaggctaccgctaaatactttttttattccaacattatgaatttttttaagaccgaaataactctcgcgaatggtgaaatccgtaaacggcctcttatagaaaccaatggtgaaacgggagaaatcgtttgggataaaggtcgtgactttgccaccgttcgtaaagtcctctcaatgccgcaagttaacattgtcaagaagacggaagttcaaacagggggattctccaaagaatctatcctgccgaagcgtaacagtgataaacttattgccagaaaaaaagattgggatccaaaaaaatacggaggctttgattcccctaccgtcgcgtatagtgtgctggtggttgctaaagtcgagaaagggaaaagcaagaaattgaaatcagttaaagaactgctgggtattacaattatggaaagatcgtcctttgagaaaaatccgatcgactttttagaggccaaggggtataaggaagtgaaaaaagatctcatcatcaaattaccgaagtatagtctttttgagctggaaaacggcagaaaaagaatgctggcctccgcgggcgagttacagaagggaaatgagctggcgctgccttccaaatatgttaattttctgtaccttgccagtcattatgagaaactgaagggcagccccgaagataacgaacagaaacaattattcgtggaacagcataagcactatttagatgaaattatagagcaaattagtgaattttctaagcgcgttatcctcgcggatgctaatttagacaaagtactgtcagcttataataaacatcgggataagccgattagagaacaggccgaaaatatcattcatttgtttaccttaaccaaccttggagcaccagctgccttcaaatatttcgataccacaattgatcgtaaacggtatacaagtacaaaagaagtcttggacgcaaccctcattcatcaatctattactggattatatgagacacgcattgatctttcacagctgggcggagac

SEQ ID NO: 66 - protein, 1368 aa, Artificial Sequence
  protein expressed from synthetic construct
MDKKYSIGLAIGTNSVGWAVITDEYKVPSKKFKVLGNTDRHSIKKNLIGALLFDSGETAEATRLKRTARRRYTRRKNRICYLQEIFSNEMAKVDDSFFHRLEESFLVEEDKKHERHPIFGNIVDEVAYHEKYPTIYHLRKKLVDSTDKADLRLIYLALAHMIKFRGHFLIEGDLNPDNSDVDKLFIQLVQTYNQLFEENPINASGVDAKAILSARLSKSRRLENLIAQLPGEKKNGLFGNLIALSLGLTPNFKSNFDLAEDAKLQLSKDTYDDDLDNLLAQIGDQYADLFLAAKNLSDAILLSDILRVNTEITKAPLSASMIKRYDEHHQDLTLLKALVRQQLPEKYKEIFFDQSKNGYAGYIDGGASQEEFYKFIKPILEKMDGTEELLVKLNREDLLRKQRTFDNGSIPHQIHLGELHAILRRQEDFYPFLKDNREKIEKILTFRIPYYVGPLARGNSRFAWMTRKSEETITPWNFEEVVDKGASAQSFIERMTNFDKNLPNEKVLPKHSLLYEYFTVYNELTKVKYVTEGMRKPAFLSGEQKKAIVDLLFKTNRKVTVKQLKEDYFKKIECFDSVEISGVEDRFNASLGTYHDLLKIIKDKDFLDNEENEDILEDIVLTLTLFEDREMIEERLKTYAHLFDDKVMKQLKRRRYTGWGRLSRKLINGIRDKQSGKTILDFLKSDGFANRNFMQLIHDDSLTFKEDIQKAQVSGQGDSLHEHIANLAGSPAIKKGILQTVKVVDELVKVMGRHKPENIVIEMARENQTTQKGQKNSRERMKRIEEGIKELGSQILKEHPVENTQLQNEKLYLYYLQNGRDMYVDQELDINRLSDYDVDHIVPQSFLKDDSIDNKVLTRSDKNRGKSDNVPSEEVVKKMKNYWRQLLNAKLITQRKFDNLTKAERGGLSELDKAGFIKRQLVETRQITKHVAQILDSRMNTKYDENDKLIREVKVITLKSKLVSDFRKDFQFYKVREINNYHHAHDAYLNAVVGTALIKKYPKLESEFVYGDYKVYDVRKMIAKSEQEIGKATAKYFFYSNIMNFFKTEITLANGEIRKRPLIETNGETGEIVWDKGRDFATVRKVLSMPQVNIVKKTEVQTGGFSKESILPKRNSDKLIARKKDWDPKKYGGFDSPTVAYSVLVVAKVEKGKSKKLKSVKELLGITIMERSSFEKNPIDFLEAKGYKEVKKDLIIKLPKYSLFELENGRKRMLASAGELQKGNELALPSKYVNFLYLASHYEKLKGSPEDNEQKQLFVEQHKHYLDEIIEQISEFSKRVILADANLDKVLSAYNKHRDKPIREQAENIIHLFTLTNLGAPAAFKYFDTTIDRKRYTSTKEVLDATLIHQSITGLYETRIDLSQLGGD

SEQ ID NO: 67 - protein, 46 aa, Artificial Sequence
  Synthetic sequence
MHHHHHHSSGLVPRGSGMKETAAAKFERQHMDSPDLGTDDDDKAMA

SEQ ID NO: 68 - DNA, 138 bp, Artificial Sequence
  Synthetic sequence
atgcaccatcatcatcatcattcttctggtctggtgccacgcggttctggtatgaaagaaaccgctgctgctaaattcgaacgccagcacatggacagcccagatctgggtaccgacgacgacgacaaggccatggcc

SEQ ID NO: 69 - DNA, 21 bp, SV40
ccaaaaaagaaacgcaaggtt

SEQ ID NO: 70 - DNA, 21 bp, T. reesei
aagaagaaaaaactgaaactg

SEQ ID NO: 71 - DNA, 19 bp, Artificial Sequence
  Primer
tgatgacggtgaaaacctc

SEQ ID NO: 72 - DNA, 16 bp, Artificial Sequence
  Primer
aaaagcaccgactcgg

SEQ ID NO: 73 - DNA, 45 bp, T. reesei
atgcgcaaatttaaagcgctgatgtgtgtctaatgcctccaccac

SEQ ID NO: 74 - DNA, 45 bp, T. reesei
atatggatctgcgcgcgatcgatgatcgtgctagcgctgctgttg

SEQ ID NO: 75 - DNA, 19 bp, Artificial Sequence
  Primer
ccaccacaggaaccaaacc

SEQ ID NO: 76 - DNA, 20 bp, Artificial Sequence
  Primer
ctgcgacggagggaatgacg

SEQ ID NO: 77 - DNA, 21 bp, Artificial Sequence
  Primer
gggcaggactggcaaggatgt

SEQ ID NO: 78 - DNA, 20 bp, Artificial Sequence
  Primer
gccgtcacgccaggaacaag

SEQ ID NO: 79 - DNA, 26 bp, Artificial Sequence
  Primer
gaacaatcttctttgcaatgttggtc

SEQ ID NO: 80 - DNA, 25 bp, Artificial Sequence
  Primer
gaggaagtcctgcttgtaggcaggc

SEQ ID NO: 81 - DNA, 26 bp, Artificial Sequence
  Primer
cgacagagcagtcatatggggatacg